European Patent Application EP 4 174 093 A1, published May 3, 2023. Title: Fully Humanized Bispecific Chimeric Antigen Receptor Targeting CD19 and CD22 and Use Thereof. Applicant: Nanjing IASO Biotherapeutics Co., Ltd. The sequence listing filed with the application follows.

SEQUENCE LISTING (70 sequences)

SEQ ID NO: 1 - DNA, 369 bp, Artificial Sequence
  CD19-62 VH nucleic acid sequence
atggccgaagtgcagctggtgcagtctggggcagaggtgaaaaagcccggggagtctctgaagatctcctgtaaggggtctggatacagctttaccaactcctggatcggatgggtgcgccagatgcccgggaaaggcctggagtggatgggactcatttaccctgatgactctgataccagatacagcccatccttccaaggccaggtcaccatctcagccgacagcgccatcaacaccgcctacctgcagtggagcagcctgaaggcctcggacaccgccatgtattactgtgcgcgccagtctacctacatctacggtggttactacgatacctggggtcaaggtactctggtgaccgtctcctca

SEQ ID NO: 2 - protein, 123 aa, Artificial Sequence
  CD19-62 VH protein sequence
MAEVQLVQSGAEVKKPGESLKISCKGSGYSFTNSWIGWVRQMPGKGLEWMGLIYPDDSDTRYSPSFQGQVTISADSAINTAYLQWSSLKASDTAMYYCARQSTYIYGGYYDTWGQGTLVTVSS

SEQ ID NO: 3 - DNA, 339 bp, Artificial Sequence
  CD19-62 VL nucleic acid sequence
cagtctgtcgtgacgcagccgccctcagtgtctggggccccagggcagagggtcaccatctcctgcactgggagcagctccaacatcggggcaggttatgatgtacactggtaccagcaacttccaggaacagcccccaaactcctcatctatgagaacaccaatcggccctcaggggtccctgaccgattctctggctccaagtctggcacctcagcctccctggccatcactgggctccaggctgaggatgaggctgattattactgccagtcctatgacagcagcctgagtggttggagggtgttcggcggagggaccaagctgaccgtcctaggt

SEQ ID NO: 4 - protein, 113 aa, Artificial Sequence
  CD19-62 VL protein sequence
QSVVTQPPSVSGAPGQRVTISCTGSSSNIGAGYDVHWYQQLPGTAPKLLIYENTNRPSGVPDRFSGSKSGTSASLAITGLQAEDEADYYCQSYDSSLSGWRVFGGGTKLTVLG

SEQ ID NO: 5 - DNA, 333 bp, Artificial Sequence
  CD19-78 VL nucleic acid sequence
caggctgtgctgactcagccaccctcggtgtctgaagcccccaggcagagggtcaccatctcctgttctggaagcagctccaacatcggaaataatgctgtaagctggtaccagcagctcccaggaaaggctcccaaactcctcatctattatgatgatctgctcccctcaggggtctctgaccgattctctggctccaagtctggcacctcagcctccctggccatcagtgggctccagtctgaggatgaggctgattattactgtgcagcatgggatgacagcctgaatggttgggtgttcggcggagggaccaaggtcaccgtcctaggt

SEQ ID NO: 6 - protein, 111 aa, Artificial Sequence
  CD19-78 VL protein sequence
QAVLTQPPSVSEAPRQRVTISCSGSSSNIGNNAVSWYQQLPGKAPKLLIYYDDLLPSGVSDRFSGSKSGTSASLAISGLQSEDEADYYCAAWDDSLNGWVFGGGTKVTVLG

SEQ ID NO: 7 - DNA, 363 bp, Artificial Sequence
  CD19-78 VH nucleic acid sequence
gaggtgcagctggtgcagtctggagcagaggtgaaaaagcccggggagtctctgaagatctcctgtaagggttctggatacagctttaccagctactggatcggctgggtgcgccagatgcccgggaaaggcctggagtggatggggatcatctatcctggtgactctgataccagatacagcccgtccttccaaggccaggtcaccatctcagccgacaagtccatcagcaccgcctacctgcagtggagcagcctgaaggcctcggacaccgccatgtattactgtgcgcgcctgtcttactcttggtcttcttggtactgggatttctggggtcaaggtactctggtgaccgtctcctca

SEQ ID NO: 8 - protein, 121 aa, Artificial Sequence
  CD19-78 VH protein sequence
EVQLVQSGAEVKKPGESLKISCKGSGYSFTSYWIGWVRQMPGKGLEWMGIIYPGDSDTRYSPSFQGQVTISADKSISTAYLQWSSLKASDTAMYYCARLSYSWSSWYWDFWGQGTLVTVSS

SEQ ID NO: 9 - DNA, 357 bp, Artificial Sequence
  CD22-80 VH nucleic acid sequence
caggtgcagctgcaggagtcgggcccaggactggtgaagccttcggggaccctgtccctcacctgcgctgtctctggtggctccatcagcagtagtaactggtggagttgggtccgccagcccccagggaaggggctggagtggattggggaaatctatcatagtgggagcaccaactacaacccgtccctcaagagtcgagtcaccatatcagtagacaagtccaagaaccagttctccctgaagctgagctctgtgaccgccgcggacacggcggtgtactactgcgccagacttcctggatacgagtcagctttcgacatatggggtcagggtacaatggtcaccgtcagctca

SEQ ID NO: 10 - protein, 119 aa, Artificial Sequence
  CD22-80 VH protein sequence
QVQLQESGPGLVKPSGTLSLTCAVSGGSISSSNWWSWVRQPPGKGLEWIGEIYHSGSTNYNPSLKSRVTISVDKSKNQFSLKLSSVTAADTAVYYCARLPGYESAFDIWGQGTMVTVSS

SEQ ID NO: 11 - DNA, 324 bp, Artificial Sequence
  CD22-80 VL nucleic acid sequence
gaaattgtgttgacgcagtctccaggcaccctgtctttgtctccaggggaaagagccaccctctcctgcagggccagtcagagtgttagcagcagctacttagcctggtaccagcagaaacctggccaggctcccaggctcctcatctatggtgcatccagcagggccactggcatcccagacaggttcagtggcagtgggtctgggacagacttcactctcaccatcagcagactggagcctgaagattttgcagtgtattactgtcagcaggccggactcttcccttacacttttggcggagggaccaaggttgagatcaaa

SEQ ID NO: 12 - protein, 108 aa, Artificial Sequence
  CD22-80 VL protein sequence
EIVLTQSPGTLSLSPGERATLSCRASQSVSSSYLAWYQQKPGQAPRLLIYGASSRATGIPDRFSGSGSGTDFTLTISRLEPEDFAVYYCQQAGLFPYTFGGGTKVEIK

SEQ ID NO: 13 - DNA, 351 bp, Artificial Sequence
  CD22-28 VH nucleic acid sequence
caggtgcagctgcaggagtcgggcccaggactggtgaagccttcggagaccctgtccctcacctgcactgtctctggtggctccatcagtagttactactggagctggatccggcagcccgccgggaagggactggagtggattgggcgtatctataccagtgggagcaccaactacaacccctccctcaagagtcgagtcaccatgtcagtagacacgtccaagaaccagttctccctgaagctgagctctgtgaccgccgcggacacggcggtgtactactgcgccagagacttgtacagagatggaatggacgtatggggccagggaacaactgtcaccgtcagctca

SEQ ID NO: 14 - protein, 117 aa, Artificial Sequence
  CD22-28 VH protein sequence
QVQLQESGPGLVKPSETLSLTCTVSGGSISSYYWSWIRQPAGKGLEWIGRIYTSGSTNYNPSLKSRVTMSVDTSKNQFSLKLSSVTAADTAVYYCARDLYRDGMDVWGQGTTVTVSS

SEQ ID NO: 15 - DNA, 321 bp, Artificial Sequence
  CD22-28 VL nucleic acid sequence
gacatccagatgacccagtctccttccaccctgtctgcatctgtaggagacagagtcaccatcacttgccgggccagtcagagtattagtagctggttggcctggtatcagcagaaaccagggaaagcccctaagctcctgatctccgatgcctccagtttggaaagtggggtcccatcaaggttcagcggcagtggatctgggacagaattcactctcaccatcagcagcctgcagcctgatgattttgcaacttattactgccagcaggccaatacctactctcctacttttggcggagggaccaaggttgagatcaaa

SEQ ID NO: 16 - protein, 107 aa, Artificial Sequence
  CD22-28 VL protein sequence
DIQMTQSPSTLSASVGDRVTITCRASQSISSWLAWYQQKPGKAPKLLISDASSLESGVPSRFSGSGSGTEFTLTISSLQPDDFATYYCQQANTYSPTFGGGTKVEIK

SEQ ID NO: 17 - DNA, 45 bp, Artificial Sequence
  Linker1 nucleic acid sequence
ggtggtggtggtagcggcggcggcggctctggtggtggtggatcc

SEQ ID NO: 18 - protein, 15 aa, Artificial Sequence
  Linker1 protein sequence
GGGGSGGGGSGGGGS

SEQ ID NO: 19 - DNA, 15 bp, Artificial Sequence
  Linker2 nucleic acid sequence
ggcggaggtgggtcc

SEQ ID NO: 20 - protein, 5 aa, Artificial Sequence
  Linker2 protein sequence
GGGGS

SEQ ID NO: 21 - DNA, 75 bp, Artificial Sequence
  Linker3 nucleic acid sequence
ggcggaggtgggtccggtggcgggggaagcggaggcggagggagcggaggagggggatctggaggcggtgggtct

SEQ ID NO: 22 - protein, 25 aa, Artificial Sequence
  Linker3 protein sequence
GGGGSGGGGSGGGGSGGGGSGGGGS

SEQ ID NO: 23 - DNA, 54 bp, Artificial Sequence
  Linker4 nucleic acid sequence
ggcagcaccagcggctccggcaagcctggctctggcgagggcagcacaaaggga

SEQ ID NO: 24 - protein, 18 aa, Artificial Sequence
  Linker4 protein sequence
GSTSGSGKPGSGEGSTKG

SEQ ID NO: 25 - DNA, 135 bp, Artificial Sequence
  CD8a hinge nucleic acid sequence
actactacccctgcacctaggcctcccaccccagccccaacaatcgccagccagcctctgtctctgcggcccgaagcctgtagacctgctgccggcggagccgtgcacaccagaggcctggacttcgcctgcgac

SEQ ID NO: 26 - protein, 45 aa, Artificial Sequence
  CD8a hinge protein sequence
TTTPAPRPPTPAPTIASQPLSLRPEACRPAAGGAVHTRGLDFACD

SEQ ID NO: 27 - DNA, 72 bp, Artificial Sequence
  CD8a TM nucleic acid sequence
atctacatctgggcccctctggccggcacctgtggcgtgctgctgctgagcctggtgatcaccctgtactgc

SEQ ID NO: 28 - protein, 24 aa, Artificial Sequence
  CD8a TM protein sequence
IYIWAPLAGTCGVLLLSLVITLYC

SEQ ID NO: 29 - DNA, 126 bp, Artificial Sequence
  4-1BB intracellular domain (IC) nucleic acid sequence
aaacggggcagaaagaaactcctgtatatattcaaacaaccatttatgagaccagtacaaactactcaagaggaagatggctgtagctgccgatttccagaagaagaagaaggaggatgtgaactg

SEQ ID NO: 30 - protein, 42 aa, Artificial Sequence
  4-1BB intracellular domain (IC) sequence
KRGRKKLLYIFKQPFMRPVQTTQEEDGCSCRFPEEEEGGCEL

SEQ ID NO: 31 - DNA, 336 bp, Artificial Sequence
  CD3z intracellular signaling domain nucleic acid sequence
agagtgaagttcagcagatccgccgacgcccctgcctaccagcagggacagaaccagctgtacaacgagctgaacctgggcagacgggaagagtacgacgtgctggacaagcggagaggccgggaccccgagatgggcggaaagcccagacggaagaacccccaggaaggcctgtataacgaactgcagaaagacaagatggccgaggcctacagcgagatcggcatgaagggcgagcggaggcgcggcaagggccacgatggcctgtaccagggcctgagcaccgccaccaaggacacctacgacgccctgcacatgcaggccctgccccccaga

SEQ ID NO: 32 - protein, 112 aa, Artificial Sequence
  CD3z intracellular signaling domain sequence
RVKFSRSADAPAYQQGQNQLYNELNLGRREEYDVLDKRRGRDPEMGGKPRRKNPQEGLYNELQKDKMAEAYSEIGMKGERRRGKGHDGLYQGLSTATKDTYDALHMQALPPR

SEQ ID NO: 33 - DNA, 54 bp, Artificial Sequence
  T2A nucleic acid sequence
gagggaaggggcagcttattaacatgtggcgatgtggaagagaaccccggtccc

SEQ ID NO: 34 - protein, 18 aa, Artificial Sequence
  T2A protein sequence
EGRGSLLTCGDVEENPGP

SEQ ID NO: 35 - DNA, 66 bp, Artificial Sequence
  CSF2RA signal nucleic acid sequence
atgctgctgctcgtgacctctttactgttatgtgagctgccccaccccgcttttttactgatccct

SEQ ID NO: 36 - protein, 22 aa, Artificial Sequence
  CSF2RA signal protein sequence
MLLLVTSLLLCELPHPAFLLIP

SEQ ID NO: 37 - DNA, 1005 bp, Artificial Sequence
  tEGFR nucleic acid sequence
cgtaaggtgtgtaacggaatcggcattggcgagttcaaggactctttaagcatcaacgccacaaacatcaagcacttcaagaattgtacctccatcagcggcgatttacacattctccccgtggcttttcgtggcgattccttcacccacaccccccctctggacccccaagagctggacattttaaaaaccgtgaaggagatcaccggctttctgctgatccaagcttggcccgagaatcgtaccgacctccacgccttcgagaatttagagattattcgtggaaggaccaagcagcacggccagttctctttagccgtcgtgtctttaaacattaccagcctcggtttaaggtctttaaaggagattagcgacggcgacgtgatcatctccggcaacaagaacctctgctacgccaacaccatcaactggaagaagctgttcggaaccagcggccaaaagaccaagatcatcagcaatcgtggagagaactcttgtaaggccactggtcaagtttgccacgccctctgtagccccgaaggatgttggggccccgagcctagggactgtgttagctgcagaaacgtgagcagaggcagagagtgtgtggacaaatgcaatttactggaaggagagcctagggagttcgtggagaacagcgaatgtatccagtgccaccccgagtgtttacctcaagccatgaacatcacttgtaccggaaggggccccgataactgcatccaatgcgcccactacatcgacggaccccactgcgtgaaaacttgtcccgccggagtgatgggagagaataacactttagtgtggaagtacgccgacgctggccacgtctgccatctgtgccaccccaactgtacctacggctgcactggtcccggtttagagggatgtcctaccaacggccccaagatcccctccatcgccaccggaatggtgggcgctctgttattactgctggtggtggctctgggcatcggtttattcatg

SEQ ID NO: 38 - protein, 335 aa, Artificial Sequence
  tEGFR protein sequence
RKVCNGIGIGEFKDSLSINATNIKHFKNCTSISGDLHILPVAFRGDSFTHTPPLDPQELDILKTVKEITGFLLIQAWPENRTDLHAFENLEIIRGRTKQHGQFSLAVVSLNITSLGLRSLKEISDGDVIISGNKNLCYANTINWKKLFGTSGQKTKIISNRGENSCKATGQVCHALCSPEGCWGPEPRDCVSCRNVSRGRECVDKCNLLEGEPREFVENSECIQCHPECLPQAMNITCTGRGPDNCIQCAHYIDGPHCVKTCPAGVMGENNTLVWKYADAGHVCHLCHPNCTYGCTGPGLEGCPTNGPKIPSIATGMVGALLLLLVVALGIGLFM

SEQ ID NO: 39 - DNA, 2328 bp, Artificial Sequence
  1# car nucleic acid sequence
atggccctgcctgtgacagctctgctcctccctctggccctgctgctccatgccgccagaccccagtctgtcgtgacgcagccgccctcagtgtctggggccccagggcagagggtcaccatctcctgcactgggagcagctccaacatcggggcaggttatgatgtacactggtaccagcaacttccaggaacagcccccaaactcctcatctatgagaacaccaatcggccctcaggggtccctgaccgattctctggctccaagtctggcacctcagcctccctggccatcactgggctccaggctgaggatgaggctgattattactgccagtcctatgacagcagcctgagtggttggagggtgttcggcggagggaccaagctgaccgtcctaggtggtggtggtggtagcggcggcggcggctctggtggtggtggatccatggccgaagtgcagctggtgcagtctggggcagaggtgaaaaagcccggggagtctctgaagatctcctgtaaggggtctggatacagctttaccaactcctggatcggatgggtgcgccagatgcccgggaaaggcctggagtggatgggactcatttaccctgatgactctgataccagatacagcccatccttccaaggccaggtcaccatctcagccgacagcgccatcaacaccgcctacctgcagtggagcagcctgaaggcctcggacaccgccatgtattactgtgcgcgccagtctacctacatctacggtggttactacgatacctggggtcaaggtactctggtgaccgtctcctcaggcggaggtgggtccggtggcgggggaagcggaggcggagggagcggaggagggggatctggaggcggtgggtctcaggtgcagctgcaggagtcgggcccaggactggtgaagccttcggggaccctgtccctcacctgcgctgtctctggtggctccatcagcagtagtaactggtggagttgggtccgccagcccccagggaaggggctggagtggattggggaaatctatcatagtgggagcaccaactacaacccgtccctcaagagtcgagtcaccatatcagtagacaagtccaagaaccagttctccctgaagctgagctctgtgaccgccgcggacacggcggtgtactactgcgccagacttcctggatacgagtcagctttcgacatatggggtcagggtacaatggtcaccgtcagctcaggtggcgggggcagcggcggaggcggatccggaggcggagggagtgaaattgtgttgacgcagtctccaggcaccctgtctttgtctccaggggaaagagccaccctctcctgcagggccagtcagagtgttagcagcagctacttagcctggtaccagcagaaacctggccaggctcccaggctcctcatctatggtgcatccagcagggccactggcatcccagacaggttcagtggcagtgggtctgggacagacttcactctcaccatcagcagactggagcctgaagattttgcagtgtattactgtcagcaggccggactcttcccttacacttttggcggagggaccaaggttgagatcaaattcgtgcccgtgttcctgcccgccaaacctactactacccctgcacctaggcctcccaccccagccccaacaatcgccagccagcctctgtctctgcggcccgaagcctgtagacctgctgccggcggagccgtgcacaccagaggcctggacttcgcctgcgacatctacatctgggcccctctggccggcacctgtggcgtgctgctgctgagcctggtgatcaccctgtactgcaaccaccggaacaaacggggcagaaagaaactcctgtatatattcaaacaaccatttatgagaccagtacaaactactcaagaggaagatggctgtagctgccgatttccagaagaagaagaaggaggatgtgaactgagagtgaagttcagcagatccgccgacgcccctgcctaccagcagggacagaaccagctgtacaacgagctgaacctgggcagacgggaagagtacgacgtgctggacaagcggagaggccgggaccccgagatgggcggaaagcccagacggaagaacccccaggaaggcctgtataacgaactgcagaaagacaagatggccgaggcctacagcgagatcggcatgaagggcgagcggaggcgcggcaagggccacgatggcctgtaccagggcctgagcaccgccaccaaggacacctacgacgccctgcacatgcaggccctgccccccaga

SEQ ID NO: 40 - protein, 776 aa, Artificial Sequence
  1# CAR protein sequence
MALPVTALLLPLALLLHAARPQSVVTQPPSVSGAPGQRVTISCTGSSSNIGAGYDVHWYQQLPGTAPKLLIYENTNRPSGVPDRFSGSKSGTSASLAITGLQAEDEADYYCQSYDSSLSGWRVFGGGTKLTVLGGGGGSGGGGSGGGGSMAEVQLVQSGAEVKKPGESLKISCKGSGYSFTNSWIGWVRQMPGKGLEWMGLIYPDDSDTRYSPSFQGQVTISADSAINTAYLQWSSLKASDTAMYYCARQSTYIYGGYYDTWGQGTLVTVSSGGGGSGGGGSGGGGSGGGGSGGGGSQVQLQESGPGLVKPSGTLSLTCAVSGGSISSSNWWSWVRQPPGKGLEWIGEIYHSGSTNYNPSLKSRVTISVDKSKNQFSLKLSSVTAADTAVYYCARLPGYESAFDIWGQGTMVTVSSGGGGSGGGGSGGGGSEIVLTQSPGTLSLSPGERATLSCRASQSVSSSYLAWYQQKPGQAPRLLIYGASSRATGIPDRFSGSGSGTDFTLTISRLEPEDFAVYYCQQAGLFPYTFGGGTKVEIKFVPVFLPAKPTTTPAPRPPTPAPTIASQPLSLRPEACRPAAGGAVHTRGLDFACDIYIWAPLAGTCGVLLLSLVITLYCNHRNKRGRKKLLYIFKQPFMRPVQTTQEEDGCSCRFPEEEEGGCELRVKFSRSADAPAYQQGQNQLYNELNLGRREEYDVLDKRRGRDPEMGGKPRRKNPQEGLYNELQKDKMAEAYSEIGMKGERRRGKGHDGLYQGLSTATKDTYDALHMQALPPR

SEQ ID NO: 41 - DNA, 2328 bp, Artificial Sequence
  2# CAR nucleic acid sequence
atggccctgcctgtgacagctctgctcctccctctggccctgctgctccatgccgccagaccccaggtgcagctgcaggagtcgggcccaggactggtgaagccttcggggaccctgtccctcacctgcgctgtctctggtggctccatcagcagtagtaactggtggagttgggtccgccagcccccagggaaggggctggagtggattggggaaatctatcatagtgggagcaccaactacaacccgtccctcaagagtcgagtcaccatatcagtagacaagtccaagaaccagttctccctgaagctgagctctgtgaccgccgcggacacggcggtgtactactgcgccagacttcctggatacgagtcagctttcgacatatggggtcagggtacaatggtcaccgtcagctcaggtggcgggggcagcggcggaggcggatccggaggcggagggagtgaaattgtgttgacgcagtctccaggcaccctgtctttgtctccaggggaaagagccaccctctcctgcagggccagtcagagtgttagcagcagctacttagcctggtaccagcagaaacctggccaggctcccaggctcctcatctatggtgcatccagcagggccactggcatcccagacaggttcagtggcagtgggtctgggacagacttcactctcaccatcagcagactggagcctgaagattttgcagtgtattactgtcagcaggccggactcttcccttacacttttggcggagggaccaaggttgagatcaaaggcggaggtgggtccggtggcgggggaagcggaggcggagggagcggaggagggggatctggaggcggtgggtctcagtctgtcgtgacgcagccgccctcagtgtctggggccccagggcagagggtcaccatctcctgcactgggagcagctccaacatcggggcaggttatgatgtacactggtaccagcaacttccaggaacagcccccaaactcctcatctatgagaacaccaatcggccctcaggggtccctgaccgattctctggctccaagtctggcacctcagcctccctggccatcactgggctccaggctgaggatgaggctgattattactgccagtcctatgacagcagcctgagtggttggagggtgttcggcggagggaccaagctgaccgtcctaggtggtggtggtggtagcggcggcggcggctctggtggtggtggatccatggccgaagtgcagctggtgcagtctggggcagaggtgaaaaagcccggggagtctctgaagatctcctgtaaggggtctggatacagctttaccaactcctggatcggatgggtgcgccagatgcccgggaaaggcctggagtggatgggactcatttaccctgatgactctgataccagatacagcccatccttccaaggccaggtcaccatctcagccgacagcgccatcaacaccgcctacctgcagtggagcagcctgaaggcctcggacaccgccatgtattactgtgcgcgccagtctacctacatctacggtggttactacgatacctggggtcaaggtactctggtgaccgtctcctcattcgtgcccgtgttcctgcccgccaaacctactactacccctgcacctaggcctcccaccccagccccaacaatcgccagccagcctctgtctctgcggcccgaagcctgtagacctgctgccggcggagccgtgcacaccagaggcctggacttcgcctgcgacatctacatctgggcccctctggccggcacctgtggcgtgctgctgctgagcctggtgatcaccctgtactgcaaccaccggaacaaacggggcagaaagaaactcctgtatatattcaaacaaccatttatgagaccagtacaaactactcaagaggaagatggctgtagctgccgatttccagaagaagaagaaggaggatgtgaactgagagtgaagttcagcagatccgccgacgcccctgcctaccagcagggacagaaccagctgtacaacgagctgaacctgggcagacgggaagagtacgacgtgctggacaagcggagaggccgggaccccgagatgggcggaaagcccagacggaagaacccccaggaaggcctgtataacgaactgcagaaagacaagatggccgaggcctacagcgagatcggcatgaagggcgagcggaggcgcggcaagggccacgatggcctgtaccagggcctgagcaccgccaccaaggacacctacgacgccctgcacatgcaggccctgccccccaga

SEQ ID NO: 42 - protein, 776 aa, Artificial Sequence
  2# CAR protein sequence
MALPVTALLLPLALLLHAARPQVQLQESGPGLVKPSGTLSLTCAVSGGSISSSNWWSWVRQPPGKGLEWIGEIYHSGSTNYNPSLKSRVTISVDKSKNQFSLKLSSVTAADTAVYYCARLPGYESAFDIWGQGTMVTVSSGGGGSGGGGSGGGGSEIVLTQSPGTLSLSPGERATLSCRASQSVSSSYLAWYQQKPGQAPRLLIYGASSRATGIPDRFSGSGSGTDFTLTISRLEPEDFAVYYCQQAGLFPYTFGGGTKVEIKGGGGSGGGGSGGGGSGGGGSGGGGSQSVVTQPPSVSGAPGQRVTISCTGSSSNIGAGYDVHWYQQLPGTAPKLLIYENTNRPSGVPDRFSGSKSGTSASLAITGLQAEDEADYYCQSYDSSLSGWRVFGGGTKLTVLGGGGGSGGGGSGGGGSMAEVQLVQSGAEVKKPGESLKISCKGSGYSFTNSWIGWVRQMPGKGLEWMGLIYPDDSDTRYSPSFQGQVTISADSAINTAYLQWSSLKASDTAMYYCARQSTYIYGGYYDTWGQGTLVTVSSFVPVFLPAKPTTTPAPRPPTPAPTIASQPLSLRPEACRPAAGGAVHTRGLDFACDIYIWAPLAGTCGVLLLSLVITLYCNHRNKRGRKKLLYIFKQPFMRPVQTTQEEDGCSCRFPEEEEGGCELRVKFSRSADAPAYQQGQNQLYNELNLGRREEYDVLDKRRGRDPEMGGKPRRKNPQEGLYNELQKDKMAEAYSEIGMKGERRRGKGHDGLYQGLSTATKDTYDALHMQALPPR

SEQ ID NO: 43 - DNA, 2298 bp, Artificial Sequence
  3# CAR nucleic acid sequence
atggccctgcctgtgacagctctgctcctccctctggccctgctgctccatgccgccagaccccagtctgtcgtgacgcagccgccctcagtgtctggggccccagggcagagggtcaccatctcctgcactgggagcagctccaacatcggggcaggttatgatgtacactggtaccagcaacttccaggaacagcccccaaactcctcatctatgagaacaccaatcggccctcaggggtccctgaccgattctctggctccaagtctggcacctcagcctccctggccatcactgggctccaggctgaggatgaggctgattattactgccagtcctatgacagcagcctgagtggttggagggtgttcggcggagggaccaagctgaccgtcctaggtggtggtggtggtagcggcggcggcggctctggtggtggtggatccatggccgaagtgcagctggtgcagtctggggcagaggtgaaaaagcccggggagtctctgaagatctcctgtaaggggtctggatacagctttaccaactcctggatcggatgggtgcgccagatgcccgggaaaggcctggagtggatgggactcatttaccctgatgactctgataccagatacagcccatccttccaaggccaggtcaccatctcagccgacagcgccatcaacaccgcctacctgcagtggagcagcctgaaggcctcggacaccgccatgtattactgtgcgcgccagtctacctacatctacggtggttactacgatacctggggtcaaggtactctggtgaccgtctcctcaggcggaggtgggtccggtggcgggggaagcggaggcggagggagccaggtgcagctgcaggagtcgggcccaggactggtgaagccttcggggaccctgtccctcacctgcgctgtctctggtggctccatcagcagtagtaactggtggagttgggtccgccagcccccagggaaggggctggagtggattggggaaatctatcatagtgggagcaccaactacaacccgtccctcaagagtcgagtcaccatatcagtagacaagtccaagaaccagttctccctgaagctgagctctgtgaccgccgcggacacggcggtgtactactgcgccagacttcctggatacgagtcagctttcgacatatggggtcagggtacaatggtcaccgtcagctcaggtggcgggggcagcggcggaggcggatccggaggcggagggagtgaaattgtgttgacgcagtctccaggcaccctgtctttgtctccaggggaaagagccaccctctcctgcagggccagtcagagtgttagcagcagctacttagcctggtaccagcagaaacctggccaggctcccaggctcctcatctatggtgcatccagcagggccactggcatcccagacaggttcagtggcagtgggtctgggacagacttcactctcaccatcagcagactggagcctgaagattttgcagtgtattactgtcagcaggccggactcttcccttacacttttggcggagggaccaaggttgagatcaaattcgtgcccgtgttcctgcccgccaaacctactactacccctgcacctaggcctcccaccccagccccaacaatcgccagccagcctctgtctctgcggcccgaagcctgtagacctgctgccggcggagccgtgcacaccagaggcctggacttcgcctgcgacatctacatctgggcccctctggccggcacctgtggcgtgctgctgctgagcctggtgatcaccctgtactgcaaccaccggaacaaacggggcagaaagaaactcctgtatatattcaaacaaccatttatgagaccagtacaaactactcaagaggaagatggctgtagctgccgatttccagaagaagaagaaggaggatgtgaactgagagtgaagttcagcagatccgccgacgcccctgcctaccagcagggacagaaccagctgtacaacgagctgaacctgggcagacgggaagagtacgacgtgctggacaagcggagaggccgggaccccgagatgggcggaaagcccagacggaagaacccccaggaaggcctgtataacgaactgcagaaagacaagatggccgaggcctacagcgagatcggcatgaagggcgagcggaggcgcggcaagggccacgatggcctgtaccagggcctgagcaccgccaccaaggacacctacgacgccctgcacatgcaggccctgccccccaga

SEQ ID NO: 44 - protein, 766 aa, Artificial Sequence
  3# CAR protein sequence
MALPVTALLLPLALLLHAARPQSVVTQPPSVSGAPGQRVTISCTGSSSNIGAGYDVHWYQQLPGTAPKLLIYENTNRPSGVPDRFSGSKSGTSASLAITGLQAEDEADYYCQSYDSSLSGWRVFGGGTKLTVLGGGGGSGGGGSGGGGSMAEVQLVQSGAEVKKPGESLKISCKGSGYSFTNSWIGWVRQMPGKGLEWMGLIYPDDSDTRYSPSFQGQVTISADSAINTAYLQWSSLKASDTAMYYCARQSTYIYGGYYDTWGQGTLVTVSSGGGGSGGGGSGGGGSQVQLQESGPGLVKPSGTLSLTCAVSGGSISSSNWWSWVRQPPGKGLEWIGEIYHSGSTNYNPSLKSRVTISVDKSKNQFSLKLSSVTAADTAVYYCARLPGYESAFDIWGQGTMVTVSSGGGGSGGGGSGGGGSEIVLTQSPGTLSLSPGERATLSCRASQSVSSSYLAWYQQKPGQAPRLLIYGASSRATGIPDRFSGSGSGTDFTLTISRLEPEDFAVYYCQQAGLFPYTFGGGTKVEIKFVPVFLPAKPTTTPAPRPPTPAPTIASQPLSLRPEACRPAAGGAVHTRGLDFACDIYIWAPLAGTCGVLLLSLVITLYCNHRNKRGRKKLLYIFKQPFMRPVQTTQEEDGCSCRFPEEEEGGCELRVKFSRSADAPAYQQGQNQLYNELNLGRREEYDVLDKRRGRDPEMGGKPRRKNPQEGLYNELQKDKMAEAYSEIGMKGERRRGKGHDGLYQGLSTATKDTYDALHMQALPPR

SEQ ID NO: 45 - DNA, 2298 bp, Artificial Sequence
  4# CAR nucleic acid sequence
atggccctgcctgtgacagctctgctcctccctctggccctgctgctccatgccgccagaccccaggtgcagctgcaggagtcgggcccaggactggtgaagccttcggggaccctgtccctcacctgcgctgtctctggtggctccatcagcagtagtaactggtggagttgggtccgccagcccccagggaaggggctggagtggattggggaaatctatcatagtgggagcaccaactacaacccgtccctcaagagtcgagtcaccatatcagtagacaagtccaagaaccagttctccctgaagctgagctctgtgaccgccgcggacacggcggtgtactactgcgccagacttcctggatacgagtcagctttcgacatatggggtcagggtacaatggtcaccgtcagctcaggtggcgggggcagcggcggaggcggatccggaggcggagggagtgaaattgtgttgacgcagtctccaggcaccctgtctttgtctccaggggaaagagccaccctctcctgcagggccagtcagagtgttagcagcagctacttagcctggtaccagcagaaacctggccaggctcccaggctcctcatctatggtgcatccagcagggccactggcatcccagacaggttcagtggcagtgggtctgggacagacttcactctcaccatcagcagactggagcctgaagattttgcagtgtattactgtcagcaggccggactcttcccttacacttttggcggagggaccaaggttgagatcaaaggcggaggtgggtccggtggcgggggaagcggaggcggagggagccagtctgtcgtgacgcagccgccctcagtgtctggggccccagggcagagggtcaccatctcctgcactgggagcagctccaacatcggggcaggttatgatgtacactggtaccagcaacttccaggaacagcccccaaactcctcatctatgagaacaccaatcggccctcaggggtccctgaccgattctctggctccaagtctggcacctcagcctccctggccatcactgggctccaggctgaggatgaggctgattattactgccagtcctatgacagcagcctgagtggttggagggtgttcggcggagggaccaagctgaccgtcctaggtggtggtggtggtagcggcggcggcggctctggtggtggtggatccatggccgaagtgcagctggtgcagtctggggcagaggtgaaaaagcccggggagtctctgaagatctcctgtaaggggtctggatacagctttaccaactcctggatcggatgggtgcgccagatgcccgggaaaggcctggagtggatgggactcatttaccctgatgactctgataccagatacagcccatccttccaaggccaggtcaccatctcagccgacagcgccatcaacaccgcctacctgcagtggagcagcctgaaggcctcggacaccgccatgtattactgtgcgcgccagtctacctacatctacggtggttactacgatacctggggtcaaggtactctggtgaccgtctcctcattcgtgcccgtgttcctgcccgccaaacctactactacccctgcacctaggcctcccaccccagccccaacaatcgccagccagcctctgtctctgcggcccgaagcctgtagacctgctgccggcggagccgtgcacaccagaggcctggacttcgcctgcgacatctacatctgggcccctctggccggcacctgtggcgtgctgctgctgagcctggtgatcaccctgtactgcaaccaccggaacaaacggggcagaaagaaactcctgtatatattcaaacaaccatttatgagaccagtacaaactactcaagaggaagatggctgtagctgccgatttccagaagaagaagaaggaggatgtgaactgagagtgaagttcagcagatccgccgacgcccctgcctaccagcagggacagaaccagctgtacaacgagctgaacctgggcagacgggaagagtacgacgtgctggacaagcggagaggccgggaccccgagatgggcggaaagcccagacggaagaacccccaggaaggcctgtataacgaactgcagaaagacaagatggccgaggcctacagcgagatcggcatgaagggcgagcggaggcgcggcaagggccacgatggcctgtaccagggcctgagcaccgccaccaaggacacctacgacgccctgcacatgcaggccctgccccccaga

SEQ ID NO: 46 - protein, 766 aa, Artificial Sequence
  4# CAR protein sequence
MALPVTALLLPLALLLHAARPQVQLQESGPGLVKPSGTLSLTCAVSGGSISSSNWWSWVRQPPGKGLEWIGEIYHSGSTNYNPSLKSRVTISVDKSKNQFSLKLSSVTAADTAVYYCARLPGYESAFDIWGQGTMVTVSSGGGGSGGGGSGGGGSEIVLTQSPGTLSLSPGERATLSCRASQSVSSSYLAWYQQKPGQAPRLLIYGASSRATGIPDRFSGSGSGTDFTLTISRLEPEDFAVYYCQQAGLFPYTFGGGTKVEIKGGGGSGGGGSGGGGSQSVVTQPPSVSGAPGQRVTISCTGSSSNIGAGYDVHWYQQLPGTAPKLLIYENTNRPSGVPDRFSGSKSGTSASLAITGLQAEDEADYYCQSYDSSLSGWRVFGGGTKLTVLGGGGGSGGGGSGGGGSMAEVQLVQSGAEVKKPGESLKISCKGSGYSFTNSWIGWVRQMPGKGLEWMGLIYPDDSDTRYSPSFQGQVTISADSAINTAYLQWSSLKASDTAMYYCARQSTYIYGGYYDTWGQGTLVTVSSFVPVFLPAKPTTTPAPRPPTPAPTIASQPLSLRPEACRPAAGGAVHTRGLDFACDIYIWAPLAGTCGVLLLSLVITLYCNHRNKRGRKKLLYIFKQPFMRPVQTTQEEDGCSCRFPEEEEGGCELRVKFSRSADAPAYQQGQNQLYNELNLGRREEYDVLDKRRGRDPEMGGKPRRKNPQEGLYNELQKDKMAEAYSEIGMKGERRRGKGHDGLYQGLSTATKDTYDALHMQALPPR

SEQ ID NO: 47 - DNA, 2268 bp, Artificial Sequence
  5# CAR nucleic acid sequence
atggccctgcctgtgacagctctgctcctccctctggccctgctgctccatgccgccagaccccagtctgtcgtgacgcagccgccctcagtgtctggggccccagggcagagggtcaccatctcctgcactgggagcagctccaacatcggggcaggttatgatgtacactggtaccagcaacttccaggaacagcccccaaactcctcatctatgagaacaccaatcggccctcaggggtccctgaccgattctctggctccaagtctggcacctcagcctccctggccatcactgggctccaggctgaggatgaggctgattattactgccagtcctatgacagcagcctgagtggttggagggtgttcggcggagggaccaagctgaccgtcctaggtggtggtggtggtagcggcggcggcggctctggtggtggtggatccatggccgaagtgcagctggtgcagtctggggcagaggtgaaaaagcccggggagtctctgaagatctcctgtaaggggtctggatacagctttaccaactcctggatcggatgggtgcgccagatgcccgggaaaggcctggagtggatgggactcatttaccctgatgactctgataccagatacagcccatccttccaaggccaggtcaccatctcagccgacagcgccatcaacaccgcctacctgcagtggagcagcctgaaggcctcggacaccgccatgtattactgtgcgcgccagtctacctacatctacggtggttactacgatacctggggtcaaggtactctggtgaccgtctcctcaggcggaggtgggtcccaggtgcagctgcaggagtcgggcccaggactggtgaagccttcggggaccctgtccctcacctgcgctgtctctggtggctccatcagcagtagtaactggtggagttgggtccgccagcccccagggaaggggctggagtggattggggaaatctatcatagtgggagcaccaactacaacccgtccctcaagagtcgagtcaccatatcagtagacaagtccaagaaccagttctccctgaagctgagctctgtgaccgccgcggacacggcggtgtactactgcgccagacttcctggatacgagtcagctttcgacatatggggtcagggtacaatggtcaccgtcagctcaggtggcgggggcagcggcggaggcggatccggaggcggagggagtgaaattgtgttgacgcagtctccaggcaccctgtctttgtctccaggggaaagagccaccctctcctgcagggccagtcagagtgttagcagcagctacttagcctggtaccagcagaaacctggccaggctcccaggctcctcatctatggtgcatccagcagggccactggcatcccagacaggttcagtggcagtgggtctgggacagacttcactctcaccatcagcagactggagcctgaagattttgcagtgtattactgtcagcaggccggactcttcccttacacttttggcggagggaccaaggttgagatcaaattcgtgcccgtgttcctgcccgccaaacctactactacccctgcacctaggcctcccaccccagccccaacaatcgccagccagcctctgtctctgcggcccgaagcctgtagacctgctgccggcggagccgtgcacaccagaggcctggacttcgcctgcgacatctacatctgggcccctctggccggcacctgtggcgtgctgctgctgagcctggtgatcaccctgtactgcaaccaccggaacaaacggggcagaaagaaactcctgtatatattcaaacaaccatttatgagaccagtacaaactactcaagaggaagatggctgtagctgccgatttccagaagaagaagaaggaggatgtgaactgagagtgaagttcagcagatccgccgacgcccctgcctaccagcagggacagaaccagctgtacaacgagctgaacctgggcagacgggaagagtacgacgtgctggacaagcggagaggccgggaccccgagatgggcggaaagcccagacggaagaacccccaggaaggcctgtataacgaactgcagaaagacaagatggccgaggcctacagcgagatcggcatgaagggcgagcggaggcgcggcaagggccacgatggcctgtaccagggcctgagcaccgccaccaaggacacctacgacgccctgcacatgcaggccctgccccccaga

SEQ ID NO: 48 - protein, 756 aa, Artificial Sequence
  5# CAR protein sequence
MALPVTALLLPLALLLHAARPQSVVTQPPSVSGAPGQRVTISCTGSSSNIGAGYDVHWYQQLPGTAPKLLIYENTNRPSGVPDRFSGSKSGTSASLAITGLQAEDEADYYCQSYDSSLSGWRVFGGGTKLTVLGGGGGSGGGGSGGGGSMAEVQLVQSGAEVKKPGESLKISCKGSGYSFTNSWIGWVRQMPGKGLEWMGLIYPDDSDTRYSPSFQGQVTISADSAINTAYLQWSSLKASDTAMYYCARQSTYIYGGYYDTWGQGTLVTVSSGGGGSQVQLQESGPGLVKPSGTLSLTCAVSGGSISSSNWWSWVRQPPGKGLEWIGEIYHSGSTNYNPSLKSRVTISVDKSKNQFSLKLSSVTAADTAVYYCARLPGYESAFDIWGQGTMVTVSSGGGGSGGGGSGGGGSEIVLTQSPGTLSLSPGERATLSCRASQSVSSSYLAWYQQKPGQAPRLLIYGASSRATGIPDRFSGSGSGTDFTLTISRLEPEDFAVYYCQQAGLFPYTFGGGTKVEIKFVPVFLPAKPTTTPAPRPPTPAPTIASQPLSLRPEACRPAAGGAVHTRGLDFACDIYIWAPLAGTCGVLLLSLVITLYCNHRNKRGRKKLLYIFKQPFMRPVQTTQEEDGCSCRFPEEEEGGCELRVKFSRSADAPAYQQGQNQLYNELNLGRREEYDVLDKRRGRDPEMGGKPRRKNPQEGLYNELQKDKMAEAYSEIGMKGERRRGKGHDGLYQGLSTATKDTYDALHMQALPPR

SEQ ID NO: 49 - DNA, 2268 bp, Artificial Sequence
  6# CAR nucleic acid sequence
atggccctgcctgtgacagctctgctcctccctctggccctgctgctccatgccgccagaccccaggtgcagctgcaggagtcgggcccaggactggtgaagccttcggggaccctgtccctcacctgcgctgtctctggtggctccatcagcagtagtaactggtggagttgggtccgccagcccccagggaaggggctggagtggattggggaaatctatcatagtgggagcaccaactacaacccgtccctcaagagtcgagtcaccatatcagtagacaagtccaagaaccagttctccctgaagctgagctctgtgaccgccgcggacacggcggtgtactactgcgccagacttcctggatacgagtcagctttcgacatatggggtcagggtacaatggtcaccgtcagctcaggtggcgggggcagcggcggaggcggatccggaggcggagggagtgaaattgtgttgacgcagtctccaggcaccctgtctttgtctccaggggaaagagccaccctctcctgcagggccagtcagagtgttagcagcagctacttagcctggtaccagcagaaacctggccaggctcccaggctcctcatctatggtgcatccagcagggccactggcatcccagacaggttcagtggcagtgggtctgggacagacttcactctcaccatcagcagactggagcctgaagattttgcagtgtattactgtcagcaggccggactcttcccttacacttttggcggagggaccaaggttgagatcaaaggcggaggtgggtcccagtctgtcgtgacgcagccgccctcagtgtctggggccccagggcagagggtcaccatctcctgcactgggagcagctccaacatcggggcaggttatgatgtacactggtaccagcaacttccaggaacagcccccaaactcctcatctatgagaacaccaatcggccctcaggggtccctgaccgattctctggctccaagtctggcacctcagcctccctggccatcactgggctccaggctgaggatgaggctgattattactgccagtcctatgacagcagcctgagtggttggagggtgttcggcggagggaccaagctgaccgtcctaggtggtggtggtggtagcggcggcggcggctctggtggtggtggatccatggccgaagtgcagctggtgcagtctggggcagaggtgaaaaagcccggggagtctctgaagatctcctgtaaggggtctggatacagctttaccaactcctggatcggatgggtgcgccagatgcccgggaaaggcctggagtggatgggactcatttaccctgatgactctgataccagatacagcccatccttccaaggccaggtcaccatctcagccgacagcgccatcaacaccgcctacctgcagtggagcagcctgaaggcctcggacaccgccatgtattactgtgcgcgccagtctacctacatctacggtggttactacgatacctggggtcaaggtactctggtgaccgtctcctcattcgtgcccgtgttcctgcccgccaaacctactactacccctgcacctaggcctcccaccccagccccaacaatcgccagccagcctctgtctctgcggcccgaagcctgtagacctgctgccggcggagccgtgcacaccagaggcctggacttcgcctgcgacatctacatctgggcccctctggccggcacctgtggcgtgctgctgctgagcctggtgatcaccctgtactgcaaccaccggaacaaacggggcagaaagaaactcctgtatatattcaaacaaccatttatgagaccagtacaaactactcaagaggaagatggctgtagctgccgatttccagaagaagaagaaggaggatgtgaactgagagtgaagttcagcagatccgccgacgcccctgcctaccagcagggacagaaccagctgtacaacgagctgaacctgggcagacgggaagagtacgacgtgctggacaagcggagaggccgggaccccgagatgggcggaaagcccagacggaagaacccccaggaaggcctgtataacgaactgcagaaagacaagatggccgaggcctacagcgagatcggcatgaagggcgagcggaggcgcggcaagggccacgatggcctgtaccagggcctgagcaccgccaccaaggacacctacgacgccctgcacatgcaggccctgccccccaga

SEQ ID NO: 50 - protein, 756 aa, Artificial Sequence
  6# CAR protein sequence
MALPVTALLLPLALLLHAARPQVQLQESGPGLVKPSGTLSLTCAVSGGSISSSNWWSWVRQPPGKGLEWIGEIYHSGSTNYNPSLKSRVTISVDKSKNQFSLKLSSVTAADTAVYYCARLPGYESAFDIWGQGTMVTVSSGGGGSGGGGSGGGGSEIVLTQSPGTLSLSPGERATLSCRASQSVSSSYLAWYQQKPGQAPRLLIYGASSRATGIPDRFSGSGSGTDFTLTISRLEPEDFAVYYCQQAGLFPYTFGGGTKVEIKGGGGSQSVVTQPPSVSGAPGQRVTISCTGSSSNIGAGYDVHWYQQLPGTAPKLLIYENTNRPSGVPDRFSGSKSGTSASLAITGLQAEDEADYYCQSYDSSLSGWRVFGGGTKLTVLGGGGGSGGGGSGGGGSMAEVQLVQSGAEVKKPGESLKISCKGSGYSFTNSWIGWVRQMPGKGLEWMGLIYPDDSDTRYSPSFQGQVTISADSAINTAYLQWSSLKASDTAMYYCARQSTYIYGGYYDTWGQGTLVTVSSFVPVFLPAKPTTTPAPRPPTPAPTIASQPLSLRPEACRPAAGGAVHTRGLDFACDIYIWAPLAGTCGVLLLSLVITLYCNHRNKRGRKKLLYIFKQPFMRPVQTTQEEDGCSCRFPEEEEGGCELRVKFSRSADAPAYQQGQNQLYNELNLGRREEYDVLDKRRGRDPEMGGKPRRKNPQEGLYNELQKDKMAEAYSEIGMKGERRRGKGHDGLYQGLSTATKDTYDALHMQALPPR

SEQ ID NO: 51 - DNA, 2259 bp, Artificial Sequence
  7# CAR nucleic acid sequence
atggccctgcctgtgacagctctgctcctccctctggccctgctgctccatgccgccagaccccagtctgtcgtgacgcagccgccctcagtgtctggggccccagggcagagggtcaccatctcctgcactgggagcagctccaacatcggggcaggttatgatgtacactggtaccagcaacttccaggaacagcccccaaactcctcatctatgagaacaccaatcggccctcaggggtccctgaccgattctctggctccaagtctggcacctcagcctccctggccatcactgggctccaggctgaggatgaggctgattattactgccagtcctatgacagcagcctgagtggttggagggtgttcggcggagggaccaagctgaccgtcctaggtggtggtggtggtagcggcggcggcggctctggtggtggtggatccatggccgaagtgcagctggtgcagtctggggcagaggtgaaaaagcccggggagtctctgaagatctcctgtaaggggtctggatacagctttaccaactcctggatcggatgggtgcgccagatgcccgggaaaggcctggagtggatgggactcatttaccctgatgactctgataccagatacagcccatccttccaaggccaggtcaccatctcagccgacagcgccatcaacaccgcctacctgcagtggagcagcctgaaggcctcggacaccgccatgtattactgtgcgcgccagtctacctacatctacggtggttactacgatacctggggtcaaggtactctggtgaccgtctcctcaggcggaggtgggtcccaggtgcagctgcaggagtcgggcccaggactggtgaagccttcggagaccctgtccctcacctgcactgtctctggtggctccatcagtagttactactggagctggatccggcagcccgccgggaagggactggagtggattgggcgtatctataccagtgggagcaccaactacaacccctccctcaagagtcgagtcaccatgtcagtagacacgtccaagaaccagttctccctgaagctgagctctgtgaccgccgcggacacggcggtgtactactgcgccagagacttgtacagagatggaatggacgtatggggccagggaacaactgtcaccgtcagctcaggtggcgggggcagcggcggaggcggatccggaggcggagggagtgacatccagatgacccagtctccttccaccctgtctgcatctgtaggagacagagtcaccatcacttgccgggccagtcagagtattagtagctggttggcctggtatcagcagaaaccagggaaagcccctaagctcctgatctccgatgcctccagtttggaaagtggggtcccatcaaggttcagcggcagtggatctgggacagaattcactctcaccatcagcagcctgcagcctgatgattttgcaacttattactgccagcaggccaatacctactctcctacttttggcggagggaccaaggttgagatcaaattcgtgcccgtgttcctgcccgccaaacctactactacccctgcacctaggcctcccaccccagccccaacaatcgccagccagcctctgtctctgcggcccgaagcctgtagacctgctgccggcggagccgtgcacaccagaggcctggacttcgcctgcgacatctacatctgggcccctctggccggcacctgtggcgtgctgctgctgagcctggtgatcaccctgtactgcaaccaccggaacaaacggggcagaaagaaactcctgtatatattcaaacaaccatttatgagaccagtacaaactactcaagaggaagatggctgtagctgccgatttccagaagaagaagaaggaggatgtgaactgagagtgaagttcagcagatccgccgacgcccctgcctaccagcagggacagaaccagctgtacaacgagctgaacctgggcagacgggaagagtacgacgtgctggacaagcggagaggccgggaccccgagatgggcggaaagcccagacggaagaacccccaggaaggcctgtataacgaactgcagaaagacaagatggccgaggcctacagcgagatcggcatgaagggcgagcggaggcgcggcaagggccacgatggcctgtaccagggcctgagcaccgccaccaaggacacctacgacgccctgcacatgcaggccctgccccccaga

SEQ ID NO: 52 - protein, 753 aa, Artificial Sequence
  7# CAR protein sequence
MALPVTALLLPLALLLHAARPQSVVTQPPSVSGAPGQRVTISCTGSSSNIGAGYDVHWYQQLPGTAPKLLIYENTNRPSGVPDRFSGSKSGTSASLAITGLQAEDEADYYCQSYDSSLSGWRVFGGGTKLTVLGGGGGSGGGGSGGGGSMAEVQLVQSGAEVKKPGESLKISCKGSGYSFTNSWIGWVRQMPGKGLEWMGLIYPDDSDTRYSPSFQGQVTISADSAINTAYLQWSSLKASDTAMYYCARQSTYIYGGYYDTWGQGTLVTVSSGGGGSQVQLQESGPGLVKPSETLSLTCTVSGGSISSYYWSWIRQPAGKGLEWIGRIYTSGSTNYNPSLKSRVTMSVDTSKNQFSLKLSSVTAADTAVYYCARDLYRDGMDVWGQGTTVTVSSGGGGSGGGGSGGGGSDIQMTQSPSTLSASVGDRVTITCRASQSISSWLAWYQQKPGKAPKLLISDASSLESGVPSRFSGSGSGTEFTLTISSLQPDDFATYYCQQANTYSPTFGGGTKVEIKFVPVFLPAKPTTTPAPRPPTPAPTIASQPLSLRPEACRPAAGGAVHTRGLDFACDIYIWAPLAGTCGVLLLSLVITLYCNHRNKRGRKKLLYIFKQPFMRPVQTTQEEDGCSCRFPEEEEGGCELRVKFSRSADAPAYQQGQNQLYNELNLGRREEYDVLDKRRGRDPEMGGKPRRKNPQEGLYNELQKDKMAEAYSEIGMKGERRRGKGHDGLYQGLSTATKDTYDALHMQALPPR

SEQ ID NO: 53 - DNA, 2259 bp, Artificial Sequence
  8# CAR nucleic acid sequence
atggccctgcctgtgacagctctgctcctccctctggccctgctgctccatgccgccagaccccaggtgcagctgcaggagtcgggcccaggactggtgaagccttcggagaccctgtccctcacctgcactgtctctggtggctccatcagtagttactactggagctggatccggcagcccgccgggaagggactggagtggattgggcgtatctataccagtgggagcaccaactacaacccctccctcaagagtcgagtcaccatgtcagtagacacgtccaagaaccagttctccctgaagctgagctctgtgaccgccgcggacacggcggtgtactactgcgccagagacttgtacagagatggaatggacgtatggggccagggaacaactgtcaccgtcagctcaggtggcgggggcagcggcggaggcggatccggaggcggagggagtgacatccagatgacccagtctccttccaccctgtctgcatctgtaggagacagagtcaccatcacttgccgggccagtcagagtattagtagctggttggcctggtatcagcagaaaccagggaaagcccctaagctcctgatctccgatgcctccagtttggaaagtggggtcccatcaaggttcagcggcagtggatctgggacagaattcactctcaccatcagcagcctgcagcctgatgattttgcaacttattactgccagcaggccaatacctactctcctacttttggcggagggaccaaggttgagatcaaaggcggaggtgggtcccagtctgtcgtgacgcagccgccctcagtgtctggggccccagggcagagggtcaccatctcctgcactgggagcagctccaacatcggggcaggttatgatgtacactggtaccagcaacttccaggaacagcccccaaactcctcatctatgagaacaccaatcggccctcaggggtccctgaccgattctctggctccaagtctggcacctcagcctccctggccatcactgggctccaggctgaggatgaggctgattattactgccagtcctatgacagcagcctgagtggttggagggtgttcggcggagggaccaagctgaccgtcctaggtggtggtggtggtagcggcggcggcggctctggtggtggtggatccatggccgaagtgcagctggtgcagtctggggcagaggtgaaaaagcccggggagtctctgaagatctcctgtaaggggtctggatacagctttaccaactcctggatcggatgggtgcgccagatgcccgggaaaggcctggagtggatgggactcatttaccctgatgactctgataccagatacagcccatccttccaaggccaggtcaccatctcagccgacagcgccatcaacaccgcctacctgcagtggagcagcctgaaggcctcggacaccgccatgtattactgtgcgcgccagtctacctacatctacggtggttactacgatacctggggtcaaggtactctggtgaccgtctcctcattcgtgcccgtgttcctgcccgccaaacctactactacccctgcacctaggcctcccaccccagccccaacaatcgccagccagcctctgtctctgcggcccgaagcctgtagacctgctgccggcggagccgtgcacaccagaggcctggacttcgcctgcgacatctacatctgggcccctctggccggcacctgtggcgtgctgctgctgagcctggtgatcaccctgtactgcaaccaccggaacaaacggggcagaaagaaactcctgtatatattcaaacaaccatttatgagaccagtacaaactactcaagaggaagatggctgtagctgccgatttccagaagaagaagaaggaggatgtgaactgagagtgaagttcagcagatccgccgacgcccctgcctaccagcagggacagaaccagctgtacaacgagctgaacctgggcagacgggaagagtacgacgtgctggacaagcggagaggccgggaccccgagatgggcggaaagcccagacggaagaacccccaggaaggcctgtataacgaactgcagaaagacaagatggccgaggcctacagcgagatcggcatgaagggcgagcggaggcgcggcaagggccacgatggcctgtaccagggcctgagcaccgccaccaaggacacctacgacgccctgcacatgcaggccctgccccccaga

SEQ ID NO: 54 - protein, 753 aa, Artificial Sequence
  8# CAR protein sequence
MALPVTALLLPLALLLHAARPQVQLQESGPGLVKPSETLSLTCTVSGGSISSYYWSWIRQPAGKGLEWIGRIYTSGSTNYNPSLKSRVTMSVDTSKNQFSLKLSSVTAADTAVYYCARDLYRDGMDVWGQGTTVTVSSGGGGSGGGGSGGGGSDIQMTQSPSTLSASVGDRVTITCRASQSISSWLAWYQQKPGKAPKLLISDASSLESGVPSRFSGSGSGTEFTLTISSLQPDDFATYYCQQANTYSPTFGGGTKVEIKGGGGSQSVVTQPPSVSGAPGQRVTISCTGSSSNIGAGYDVHWYQQLPGTAPKLLIYENTNRPSGVPDRFSGSKSGTSASLAITGLQAEDEADYYCQSYDSSLSGWRVFGGGTKLTVLGGGGGSGGGGSGGGGSMAEVQLVQSGAEVKKPGESLKISCKGSGYSFTNSWIGWVRQMPGKGLEWMGLIYPDDSDTRYSPSFQGQVTISADSAINTAYLQWSSLKASDTAMYYCARQSTYIYGGYYDTWGQGTLVTVSSFVPVFLPAKPTTTPAPRPPTPAPTIASQPLSLRPEACRPAAGGAVHTRGLDFACDIYIWAPLAGTCGVLLLSLVITLYCNHRNKRGRKKLLYIFKQPFMRPVQTTQEEDGCSCRFPEEEEGGCELRVKFSRSADAPAYQQGQNQLYNELNLGRREEYDVLDKRRGRDPEMGGKPRRKNPQEGLYNELQKDKMAEAYSEIGMKGERRRGKGHDGLYQGLSTATKDTYDALHMQALPPR

SEQ ID NO: 55 - DNA, 2247 bp, Artificial Sequence
  9# CAR nucleic acid sequence
atggccctgcctgtgacagctctgctcctccctctggccctgctgctccatgccgccagaccccagtctgtcgtgacgcagccgccctcagtgtctggggccccagggcagagggtcaccatctcctgcactgggagcagctccaacatcggggcaggttatgatgtacactggtaccagcaacttccaggaacagcccccaaactcctcatctatgagaacaccaatcggccctcaggggtccctgaccgattctctggctccaagtctggcacctcagcctccctggccatcactgggctccaggctgaggatgaggctgattattactgccagtcctatgacagcagcctgagtggttggagggtgttcggcggagggaccaagctgaccgtcctaggtggtggtggtggtagccaggtgcagctgcaggagtcgggcccaggactggtgaagccttcggggaccctgtccctcacctgcgctgtctctggtggctccatcagcagtagtaactggtggagttgggtccgccagcccccagggaaggggctggagtggattggggaaatctatcatagtgggagcaccaactacaacccgtccctcaagagtcgagtcaccatatcagtagacaagtccaagaaccagttctccctgaagctgagctctgtgaccgccgcggacacggcggtgtactactgcgccagacttcctggatacgagtcagctttcgacatatggggtcagggtacaatggtcaccgtcagctcaggcagcaccagcggctccggcaagcctggctctggcgagggcagcacaaagggagaaattgtgttgacgcagtctccaggcaccctgtctttgtctccaggggaaagagccaccctctcctgcagggccagtcagagtgttagcagcagctacttagcctggtaccagcagaaacctggccaggctcccaggctcctcatctatggtgcatccagcagggccactggcatcccagacaggttcagtggcagtgggtctgggacagacttcactctcaccatcagcagactggagcctgaagattttgcagtgtattactgtcagcaggccggactcttcccttacacttttggcggagggaccaaggttgagatcaaaggtggcgggggcagcatggccgaagtgcagctggtgcagtctggggcagaggtgaaaaagcccggggagtctctgaagatctcctgtaaggggtctggatacagctttaccaactcctggatcggatgggtgcgccagatgcccgggaaaggcctggagtggatgggactcatttaccctgatgactctgataccagatacagcccatccttccaaggccaggtcaccatctcagccgacagcgccatcaacaccgcctacctgcagtggagcagcctgaaggcctcggacaccgccatgtattactgtgcgcgccagtctacctacatctacggtggttactacgatacctggggtcaaggtactctggtgaccgtctcctcattcgtgcccgtgttcctgcccgccaaacctactactacccctgcacctaggcctcccaccccagccccaacaatcgccagccagcctctgtctctgcggcccgaagcctgtagacctgctgccggcggagccgtgcacaccagaggcctggacttcgcctgcgacatctacatctgggcccctctggccggcacctgtggcgtgctgctgctgagcctggtgatcaccctgtactgcaaccaccggaacaaacggggcagaaagaaactcctgtatatattcaaacaaccatttatgagaccagtacaaactactcaagaggaagatggctgtagctgccgatttccagaagaagaagaaggaggatgtgaactgagagtgaagttcagcagatccgccgacgcccctgcctaccagcagggacagaaccagctgtacaacgagctgaacctgggcagacgggaagagtacgacgtgctggacaagcggagaggccgggaccccgagatgggcggaaagcccagacggaagaacccccaggaaggcctgtataacgaactgcagaaagacaagatggccgaggcctacagcgagatcggcatgaagggcgagcggaggcgcggcaagggccacgatggcctgtaccagggcctgagcaccgccaccaaggacacctacgacgccctgcacatgcaggccctgccccccaga

SEQ ID NO: 56 - protein, 749 aa, Artificial Sequence
  9# CAR protein sequence
MALPVTALLLPLALLLHAARPQSVVTQPPSVSGAPGQRVTISCTGSSSNIGAGYDVHWYQQLPGTAPKLLIYENTNRPSGVPDRFSGSKSGTSASLAITGLQAEDEADYYCQSYDSSLSGWRVFGGGTKLTVLGGGGGSQVQLQESGPGLVKPSGTLSLTCAVSGGSISSSNWWSWVRQPPGKGLEWIGEIYHSGSTNYNPSLKSRVTISVDKSKNQFSLKLSSVTAADTAVYYCARLPGYESAFDIWGQGTMVTVSSGSTSGSGKPGSGEGSTKGEIVLTQSPGTLSLSPGERATLSCRASQSVSSSYLAWYQQKPGQAPRLLIYGASSRATGIPDRFSGSGSGTDFTLTISRLEPEDFAVYYCQQAGLFPYTFGGGTKVEIKGGGGSMAEVQLVQSGAEVKKPGESLKISCKGSGYSFTNSWIGWVRQMPGKGLEWMGLIYPDDSDTRYSPSFQGQVTISADSAINTAYLQWSSLKASDTAMYYCARQSTYIYGGYYDTWGQGTLVTVSSFVPVFLPAKPTTTPAPRPPTPAPTIASQPLSLRPEACRPAAGGAVHTRGLDFACDIYIWAPLAGTCGVLLLSLVITLYCNHRNKRGRKKLLYIFKQPFMRPVQTTQEEDGCSCRFPEEEEGGCELRVKFSRSADAPAYQQGQNQLYNELNLGRREEYDVLDKRRGRDPEMGGKPRRKNPQEGLYNELQKDKMAEAYSEIGMKGERRRGKGHDGLYQGLSTATKDTYDALHMQALPPR

SEQ ID NO: 57 - DNA, 2238 bp, Artificial Sequence
  10# CAR nucleic acid sequence
atggccctgcctgtgacagctctgctcctccctctggccctgctgctccatgccgccagaccccagtctgtcgtgacgcagccgccctcagtgtctggggccccagggcagagggtcaccatctcctgcactgggagcagctccaacatcggggcaggttatgatgtacactggtaccagcaacttccaggaacagcccccaaactcctcatctatgagaacaccaatcggccctcaggggtccctgaccgattctctggctccaagtctggcacctcagcctccctggccatcactgggctccaggctgaggatgaggctgattattactgccagtcctatgacagcagcctgagtggttggagggtgttcggcggagggaccaagctgaccgtcctaggtggtggtggtggtagccaggtgcagctgcaggagtcgggcccaggactggtgaagccttcggagaccctgtccctcacctgcactgtctctggtggctccatcagtagttactactggagctggatccggcagcccgccgggaagggactggagtggattgggcgtatctataccagtgggagcaccaactacaacccctccctcaagagtcgagtcaccatgtcagtagacacgtccaagaaccagttctccctgaagctgagctctgtgaccgccgcggacacggcggtgtactactgcgccagagacttgtacagagatggaatggacgtatggggccagggaacaactgtcaccgtcagctcaggcagcaccagcggctccggcaagcctggctctggcgagggcagcacaaagggagacatccagatgacccagtctccttccaccctgtctgcatctgtaggagacagagtcaccatcacttgccgggccagtcagagtattagtagctggttggcctggtatcagcagaaaccagggaaagcccctaagctcctgatctccgatgcctccagtttggaaagtggggtcccatcaaggttcagcggcagtggatctgggacagaattcactctcaccatcagcagcctgcagcctgatgattttgcaacttattactgccagcaggccaatacctactctcctacttttggcggagggaccaaggttgagatcaaaggtggcgggggcagcatggccgaagtgcagctggtgcagtctggggcagaggtgaaaaagcccggggagtctctgaagatctcctgtaaggggtctggatacagctttaccaactcctggatcggatgggtgcgccagatgcccgggaaaggcctggagtggatgggactcatttaccctgatgactctgataccagatacagcccatccttccaaggccaggtcaccatctcagccgacagcgccatcaacaccgcctacctgcagtggagcagcctgaaggcctcggacaccgccatgtattactgtgcgcgccagtctacctacatctacggtggttactacgatacctggggtcaaggtactctggtgaccgtctcctcattcgtgcccgtgttcctgcccgccaaacctactactacccctgcacctaggcctcccaccccagccccaacaatcgccagccagcctctgtctctgcggcccgaagcctgtagacctgctgccggcggagccgtgcacaccagaggcctggacttcgcctgcgacatctacatctgggcccctctggccggcacctgtggcgtgctgctgctgagcctggtgatcaccctgtactgcaaccaccggaacaaacggggcagaaagaaactcctgtatatattcaaacaaccatttatgagaccagtacaaactactcaagaggaagatggctgtagctgccgatttccagaagaagaagaaggaggatgtgaactgagagtgaagttcagcagatccgccgacgcccctgcctaccagcagggacagaaccagctgtacaacgagctgaacctgggcagacgggaagagtacgacgtgctggacaagcggagaggccgggaccccgagatgggcggaaagcccagacggaagaacccccaggaaggcctgtataacgaactgcagaaagacaagatggccgaggcctacagcgagatcggcatgaagggcgagcggaggcgcggcaagggccacgatggcctgtaccagggcctgagcaccgccaccaaggacacctacgacgccctgcacatgcaggccctgccccccaga

SEQ ID NO: 58 - protein, 746 aa, Artificial Sequence
  10# CAR protein sequence
MALPVTALLLPLALLLHAARPQSVVTQPPSVSGAPGQRVTISCTGSSSNIGAGYDVHWYQQLPGTAPKLLIYENTNRPSGVPDRFSGSKSGTSASLAITGLQAEDEADYYCQSYDSSLSGWRVFGGGTKLTVLGGGGGSQVQLQESGPGLVKPSETLSLTCTVSGGSISSYYWSWIRQPAGKGLEWIGRIYTSGSTNYNPSLKSRVTMSVDTSKNQFSLKLSSVTAADTAVYYCARDLYRDGMDVWGQGTTVTVSSGSTSGSGKPGSGEGSTKGDIQMTQSPSTLSASVGDRVTITCRASQSISSWLAWYQQKPGKAPKLLISDASSLESGVPSRFSGSGSGTEFTLTISSLQPDDFATYYCQQANTYSPTFGGGTKVEIKGGGGSMAEVQLVQSGAEVKKPGESLKISCKGSGYSFTNSWIGWVRQMPGKGLEWMGLIYPDDSDTRYSPSFQGQVTISADSAINTAYLQWSSLKASDTAMYYCARQSTYIYGGYYDTWGQGTLVTVSSFVPVFLPAKPTTTPAPRPPTPAPTIASQPLSLRPEACRPAAGGAVHTRGLDFACDIYIWAPLAGTCGVLLLSLVITLYCNHRNKRGRKKLLYIFKQPFMRPVQTTQEEDGCSCRFPEEEEGGCELRVKFSRSADAPAYQQGQNQLYNELNLGRREEYDVLDKRRGRDPEMGGKPRRKNPQEGLYNELQKDKMAEAYSEIGMKGERRRGKGHDGLYQGLSTATKDTYDALHMQALPPR

SEQ ID NO: 59 - DNA, 2247 bp, Artificial Sequence
  11# CAR nucleic acid sequence
atggccctgcctgtgacagctctgctcctccctctggccctgctgctccatgccgccagacccgaaattgtgttgacgcagtctccaggcaccctgtctttgtctccaggggaaagagccaccctctcctgcagggccagtcagagtgttagcagcagctacttagcctggtaccagcagaaacctggccaggctcccaggctcctcatctatggtgcatccagcagggccactggcatcccagacaggttcagtggcagtgggtctgggacagacttcactctcaccatcagcagactggagcctgaagattttgcagtgtattactgtcagcaggccggactcttcccttacacttttggcggagggaccaaggttgagatcaaaggtggcgggggcagcatggccgaagtgcagctggtgcagtctggggcagaggtgaaaaagcccggggagtctctgaagatctcctgtaaggggtctggatacagctttaccaactcctggatcggatgggtgcgccagatgcccgggaaaggcctggagtggatgggactcatttaccctgatgactctgataccagatacagcccatccttccaaggccaggtcaccatctcagccgacagcgccatcaacaccgcctacctgcagtggagcagcctgaaggcctcggacaccgccatgtattactgtgcgcgccagtctacctacatctacggtggttactacgatacctggggtcaaggtactctggtgaccgtctcctcaggcagcaccagcggctccggcaagcctggctctggcgagggcagcacaaagggacagtctgtcgtgacgcagccgccctcagtgtctggggccccagggcagagggtcaccatctcctgcactgggagcagctccaacatcggggcaggttatgatgtacactggtaccagcaacttccaggaacagcccccaaactcctcatctatgagaacaccaatcggccctcaggggtccctgaccgattctctggctccaagtctggcacctcagcctccctggccatcactgggctccaggctgaggatgaggctgattattactgccagtcctatgacagcagcctgagtggttggagggtgttcggcggagggaccaagctgaccgtcctaggtggtggtggtggtagccaggtgcagctgcaggagtcgggcccaggactggtgaagccttcggggaccctgtccctcacctgcgctgtctctggtggctccatcagcagtagtaactggtggagttgggtccgccagcccccagggaaggggctggagtggattggggaaatctatcatagtgggagcaccaactacaacccgtccctcaagagtcgagtcaccatatcagtagacaagtccaagaaccagttctccctgaagctgagctctgtgaccgccgcggacacggcggtgtactactgcgccagacttcctggatacgagtcagctttcgacatatggggtcagggtacaatggtcaccgtcagctcattcgtgcccgtgttcctgcccgccaaacctactactacccctgcacctaggcctcccaccccagccccaacaatcgccagccagcctctgtctctgcggcccgaagcctgtagacctgctgccggcggagccgtgcacaccagaggcctggacttcgcctgcgacatctacatctgggcccctctggccggcacctgtggcgtgctgctgctgagcctggtgatcaccctgtactgcaaccaccggaacaaacggggcagaaagaaactcctgtatatattcaaacaaccatttatgagaccagtacaaactactcaagaggaagatggctgtagctgccgatttccagaagaagaagaaggaggatgtgaactgagagtgaagttcagcagatccgccgacgcccctgcctaccagcagggacagaaccagctgtacaacgagctgaacctgggcagacgggaagagtacgacgtgctggacaagcggagaggccgggaccccgagatgggcggaaagcccagacggaagaacccccaggaaggcctgtataacgaactgcagaaagacaagatggccgaggcctacagcgagatcggcatgaagggcgagcggaggcgcggcaagggccacgatggcctgtaccagggcctgagcaccgccaccaaggacacctacgacgccctgcacatgcaggccctgccccccaga

SEQ ID NO: 60 - protein, 749 aa, Artificial Sequence
  11# CAR protein sequence
MALPVTALLLPLALLLHAARPEIVLTQSPGTLSLSPGERATLSCRASQSVSSSYLAWYQQKPGQAPRLLIYGASSRATGIPDRFSGSGSGTDFTLTISRLEPEDFAVYYCQQAGLFPYTFGGGTKVEIKGGGGSMAEVQLVQSGAEVKKPGESLKISCKGSGYSFTNSWIGWVRQMPGKGLEWMGLIYPDDSDTRYSPSFQGQVTISADSAINTAYLQWSSLKASDTAMYYCARQSTYIYGGYYDTWGQGTLVTVSSGSTSGSGKPGSGEGSTKGQSVVTQPPSVSGAPGQRVTISCTGSSSNIGAGYDVHWYQQLPGTAPKLLIYENTNRPSGVPDRFSGSKSGTSASLAITGLQAEDEADYYCQSYDSSLSGWRVFGGGTKLTVLGGGGGSQVQLQESGPGLVKPSGTLSLTCAVSGGSISSSNWWSWVRQPPGKGLEWIGEIYHSGSTNYNPSLKSRVTISVDKSKNQFSLKLSSVTAADTAVYYCARLPGYESAFDIWGQGTMVTVSSFVPVFLPAKPTTTPAPRPPTPAPTIASQPLSLRPEACRPAAGGAVHTRGLDFACDIYIWAPLAGTCGVLLLSLVITLYCNHRNKRGRKKLLYIFKQPFMRPVQTTQEEDGCSCRFPEEEEGGCELRVKFSRSADAPAYQQGQNQLYNELNLGRREEYDVLDKRRGRDPEMGGKPRRKNPQEGLYNELQKDKMAEAYSEIGMKGERRRGKGHDGLYQGLSTATKDTYDALHMQALPPR

SEQ ID NO: 61 - DNA, 2238 bp, Artificial Sequence
  12# CAR nucleic acid sequence
atggccctgcctgtgacagctctgctcctccctctggccctgctgctccatgccgccagacccgacatccagatgacccagtctccttccaccctgtctgcatctgtaggagacagagtcaccatcacttgccgggccagtcagagtattagtagctggttggcctggtatcagcagaaaccagggaaagcccctaagctcctgatctccgatgcctccagtttggaaagtggggtcccatcaaggttcagcggcagtggatctgggacagaattcactctcaccatcagcagcctgcagcctgatgattttgcaacttattactgccagcaggccaatacctactctcctacttttggcggagggaccaaggttgagatcaaaggtggcgggggcagcatggccgaagtgcagctggtgcagtctggggcagaggtgaaaaagcccggggagtctctgaagatctcctgtaaggggtctggatacagctttaccaactcctggatcggatgggtgcgccagatgcccgggaaaggcctggagtggatgggactcatttaccctgatgactctgataccagatacagcccatccttccaaggccaggtcaccatctcagccgacagcgccatcaacaccgcctacctgcagtggagcagcctgaaggcctcggacaccgccatgtattactgtgcgcgccagtctacctacatctacggtggttactacgatacctggggtcaaggtactctggtgaccgtctcctcaggcagcaccagcggctccggcaagcctggctctggcgagggcagcacaaagggacagtctgtcgtgacgcagccgccctcagtgtctggggccccagggcagagggtcaccatctcctgcactgggagcagctccaacatcggggcaggttatgatgtacactggtaccagcaacttccaggaacagcccccaaactcctcatctatgagaacaccaatcggccctcaggggtccctgaccgattctctggctccaagtctggcacctcagcctccctggccatcactgggctccaggctgaggatgaggctgattattactgccagtcctatgacagcagcctgagtggttggagggtgttcggcggagggaccaagctgaccgtcctaggtggtggtggtggtagccaggtgcagctgcaggagtcgggcccaggactggtgaagccttcggagaccctgtccctcacctgcactgtctctggtggctccatcagtagttactactggagctggatccggcagcccgccgggaagggactggagtggattgggcgtatctataccagtgggagcaccaactacaacccctccctcaagagtcgagtcaccatgtcagtagacacgtccaagaaccagttctccctgaagctgagctctgtgaccgccgcggacacggcggtgtactactgcgccagagacttgtacagagatggaatggacgtatggggccagggaacaactgtcaccgtcagctcattcgtgcccgtgttcctgcccgccaaacctactactacccctgcacctaggcctcccaccccagccccaacaatcgccagccagcctctgtctctgcggcccgaagcctgtagacctgctgccggcggagccgtgcacaccagaggcctggacttcgcctgcgacatctacatctgggcccctctggccggcacctgtggcgtgctgctgctgagcctggtgatcaccctgtactgcaaccaccggaacaaacggggcagaaagaaactcctgtatatattcaaacaaccatttatgagaccagtacaaactactcaagaggaagatggctgtagctgccgatttccagaagaagaagaaggaggatgtgaactgagagtgaagttcagcagatccgccgacgcccctgcctaccagcagggacagaaccagctgtacaacgagctgaacctgggcagacgggaagagtacgacgtgctggacaagcggagaggccgggaccccgagatgggcggaaagcccagacggaagaacccccaggaaggcctgtataacgaactgcagaaagacaagatggccgaggcctacagcgagatcggcatgaagggcgagcggaggcgcggcaagggccacgatggcctgtaccagggcctgagcaccgccaccaaggacacctacgacgccctgcacatgcaggccctgccccccaga

SEQ ID NO: 62 - protein, 746 aa, Artificial Sequence
  12# CAR protein sequence
MALPVTALLLPLALLLHAARPDIQMTQSPSTLSASVGDRVTITCRASQSISSWLAWYQQKPGKAPKLLISDASSLESGVPSRFSGSGSGTEFTLTISSLQPDDFATYYCQQANTYSPTFGGGTKVEIKGGGGSMAEVQLVQSGAEVKKPGESLKISCKGSGYSFTNSWIGWVRQMPGKGLEWMGLIYPDDSDTRYSPSFQGQVTISADSAINTAYLQWSSLKASDTAMYYCARQSTYIYGGYYDTWGQGTLVTVSSGSTSGSGKPGSGEGSTKGQSVVTQPPSVSGAPGQRVTISCTGSSSNIGAGYDVHWYQQLPGTAPKLLIYENTNRPSGVPDRFSGSKSGTSASLAITGLQAEDEADYYCQSYDSSLSGWRVFGGGTKLTVLGGGGGSQVQLQESGPGLVKPSETLSLTCTVSGGSISSYYWSWIRQPAGKGLEWIGRIYTSGSTNYNPSLKSRVTMSVDTSKNQFSLKLSSVTAADTAVYYCARDLYRDGMDVWGQGTTVTVSSFVPVFLPAKPTTTPAPRPPTPAPTIASQPLSLRPEACRPAAGGAVHTRGLDFACDIYIWAPLAGTCGVLLLSLVITLYCNHRNKRGRKKLLYIFKQPFMRPVQTTQEEDGCSCRFPEEEEGGCELRVKFSRSADAPAYQQGQNQLYNELNLGRREEYDVLDKRRGRDPEMGGKPRRKNPQEGLYNELQKDKMAEAYSEIGMKGERRRGKGHDGLYQGLSTATKDTYDALHMQALPPR

SEQ ID NO: 63 - DNA, 2235 bp, Artificial Sequence
  PXL1419 CAR nucleic acid sequence
atggccctgcctgtgacagctctgctcctccctctggccctgctgctccatgccgccagaccccaggctgtgctgactcagccaccctcggtgtctgaagcccccaggcagagggtcaccatctcctgttctggaagcagctccaacatcggaaataatgctgtaagctggtaccagcagctcccaggaaaggctcccaaactcctcatctattatgatgatctgctcccctcaggggtctctgaccgattctctggctccaagtctggcacctcagcctccctggccatcagtgggctccagtctgaggatgaggctgattattactgtgcagcatgggatgacagcctgaatggttgggtgttcggcggagggaccaaggtcaccgtcctaggtggtggtggtggtagccaggtgcagctgcaggagtcgggcccaggactggtgaagccttcggggaccctgtccctcacctgcgctgtctctggtggctccatcagcagtagtaactggtggagttgggtccgccagcccccagggaaggggctggagtggattggggaaatctatcatagtgggagcaccaactacaacccgtccctcaagagtcgagtcaccatatcagtagacaagtccaagaaccagttctccctgaagctgagctctgtgaccgccgcggacacggcggtgtactactgcgccagacttcctggatacgagtcagctttcgacatatggggtcagggtacaatggtcaccgtcagctcaggcagcaccagcggctccggcaagcctggctctggcgagggcagcacaaagggagaaattgtgttgacgcagtctccaggcaccctgtctttgtctccaggggaaagagccaccctctcctgcagggccagtcagagtgttagcagcagctacttagcctggtaccagcagaaacctggccaggctcccaggctcctcatctatggtgcatccagcagggccactggcatcccagacaggttcagtggcagtgggtctgggacagacttcactctcaccatcagcagactggagcctgaagattttgcagtgtattactgtcagcaggccggactcttcccttacacttttggcggagggaccaaggttgagatcaaaggaggcggagggagtgaggtgcagctggtgcagtctggagcagaggtgaaaaagcccggggagtctctgaagatctcctgtaagggttctggatacagctttaccagctactggatcggctgggtgcgccagatgcccgggaaaggcctggagtggatggggatcatctatcctggtgactctgataccagatacagcccgtccttccaaggccaggtcaccatctcagccgacaagtccatcagcaccgcctacctgcagtggagcagcctgaaggcctcggacaccgccatgtattactgtgcgcgcctgtcttactcttggtcttcttggtactgggatttctggggtcaaggtactctggtgaccgtctcctcattcgtgcccgtgttcctgcccgccaaacctactactacccctgcacctaggcctcccaccccagccccaacaatcgccagccagcctctgtctctgcggcccgaagcctgtagacctgctgccggcggagccgtgcacaccagaggcctggacttcgcctgcgacatctacatctgggcccctctggccggcacctgtggcgtgctgctgctgagcctggtgatcaccctgtactgcaaccaccggaacaaacggggcagaaagaaactcctgtatatattcaaacaaccatttatgagaccagtacaaactactcaagaggaagatggctgtagctgccgatttccagaagaagaagaaggaggatgtgaactgagagtgaagttcagcagatccgccgacgcccctgcctaccagcagggacagaaccagctgtacaacgagctgaacctgggcagacgggaagagtacgacgtgctggacaagcggagaggccgggaccccgagatgggcggaaagcccagacggaagaacccccaggaaggcctgtataacgaactgcagaaagacaagatggccgaggcctacagcgagatcggcatgaagggcgagcggaggcgcggcaagggccacgatggcctgtaccagggcctgagcaccgccaccaaggacacctacgacgccctgcacatgcaggccctgccccccaga

SEQ ID NO: 64 - protein, 745 aa, Artificial Sequence
  PXL1419 CAR protein sequence
MALPVTALLLPLALLLHAARPQAVLTQPPSVSEAPRQRVTISCSGSSSNIGNNAVSWYQQLPGKAPKLLIYYDDLLPSGVSDRFSGSKSGTSASLAISGLQSEDEADYYCAAWDDSLNGWVFGGGTKVTVLGGGGGSQVQLQESGPGLVKPSGTLSLTCAVSGGSISSSNWWSWVRQPPGKGLEWIGEIYHSGSTNYNPSLKSRVTISVDKSKNQFSLKLSSVTAADTAVYYCARLPGYESAFDIWGQGTMVTVSSGSTSGSGKPGSGEGSTKGEIVLTQSPGTLSLSPGERATLSCRASQSVSSSYLAWYQQKPGQAPRLLIYGASSRATGIPDRFSGSGSGTDFTLTISRLEPEDFAVYYCQQAGLFPYTFGGGTKVEIKGGGGSEVQLVQSGAEVKKPGESLKISCKGSGYSFTSYWIGWVRQMPGKGLEWMGIIYPGDSDTRYSPSFQGQVTISADKSISTAYLQWSSLKASDTAMYYCARLSYSWSSWYWDFWGQGTLVTVSSFVPVFLPAKPTTTPAPRPPTPAPTIASQPLSLRPEACRPAAGGAVHTRGLDFACDIYIWAPLAGTCGVLLLSLVITLYCNHRNKRGRKKLLYIFKQPFMRPVQTTQEEDGCSCRFPEEEEGGCELRVKFSRSADAPAYQQGQNQLYNELNLGRREEYDVLDKRRGRDPEMGGKPRRKNPQEGLYNELQKDKMAEAYSEIGMKGERRRGKGHDGLYQGLSTATKDTYDALHMQALPPR

SEQ ID NO: 65 - DNA, 2235 bp, Artificial Sequence
  PXL1435 CAR nucleic acid sequence
atggcacttcctgtgacagccttgctcttgcccttagcactgctgcttcatgcggcgagacctgaggtccaacttgtgcaatcaggagcagaagtgaagaagccaggcgaatcacttaagatttcctgcaaaggatcaggatactcatttacatcatactggatcggatgggtccggcagatgcccggcaaaggattggagtggatgggcatcatctaccctggagattcagatacaagatactcaccttccttccaaggccaggtcaccatatcggctgacaaatcaatctcaacagcataccttcaatggtcatcacttaaagcatcagatacagcaatgtactactgcgcaaggcttagctattcatggtcatcatggtactgggatttctgggggcaaggcacgctggttacagtctcatccggagggggagggagcgagatcgtcctcactcagtctccaggcaccctgtctttgtcacctggagaacgggcaacactttcatgcagagcatcacaaagcgttagtagtagctatcttgcctggtatcagcaaaaaccgggccaggcacctagactgctcatttatggagcttcctcaagagcaacaggaatccctgaccggttcagcgggtccggctctggtactgatttcaccttaacaatctcaagacttgaacctgaagatttcgcagtgtattattgtcagcaggcaggactcttcccgtatacattcggcggaggcacaaaagtggaaattaaaggtagtacctccggatcaggaaagccgggctctggagaaggatctacaaagggccaggttcaacttcaagaatccggcccaggtttggtaaagccttcaggtaccttatcgctgacttgtgcagtgtcaggaggatcaatctccagtagtaattggtggtcatgggtccgacagcctccagggaaaggactagagtggattggcgagatttaccactctgggagtaccaactacaacccttcacttaaatcacgagtcacaattagtgttgataaatcaaagaatcaattcagcctcaagctatcatcagtgacagcagcagatacagcggtctattattgtgctagacttccaggctacgaatcagcatttgatatctggggacaaggaaccatggtaactgttagtagcggaggaggtggctcccaagcagtactgacgcagccgccctcagtgtcagaggcgccaaggcaaagagtaaccataagttgttctggatcttccagcaatattggtaacaacgcagtgagctggtatcagcagctaccgggaaaggctcccaagctattgatatattatgacgatcttcttccttcaggagtgtcagacaggttctcgggttctaaatcaggcacatcagcatcacttgccatcagcggcctgcagagcgaagatgaagcagattattattgtgccgcgtgggatgattcacttaacggatgggtgttcggcggaggcacgaaggtgacagtacttggttttgtacctgtgtttcttcctgcaaagccgaccacaactcccgcacctagacctccaactccggcaccaaccattgcatcacaacctctaagtctgaggcccgaggcatgcagacctgcagcaggaggagcagtgcacacaagaggacttgatttcgcgtgtgatatctacatctgggcacccctggccggaacatgtggagtgcttcttctttcacttgtgatcacactttactgcaaccacagaaacaagcgcggtagaaagaagctactgtacatctttaaacaacctttcatgcgtcctgtgcaaacaacacaagaagaagatggatgctcatgcagatttcctgaagaagaagaaggaggatgcgaacttagagtgaaattcagccgatcagcagatgcacctgcataccaacaaggacagaatcagctctataatgagctgaatttgggaagaagagaagaatacgatgtgcttgataagcgcagaggtcgagacccagaaatgggaggaaagccgaggaggaagaatccgcaagaaggactatataatgagctccagaaggataagatggctgaagcatactcagaaatcggaatgaaaggagaaagaagaagaggaaagggccatgatggactttaccaaggactttcaacagcaacaaaggacacttacgatgcacttcacatgcaagcacttcctcctaga

SEQ ID NO: 66 - protein, 745 aa, Artificial Sequence
  PXL1435 CAR protein sequence
MALPVTALLLPLALLLHAARPEVQLVQSGAEVKKPGESLKISCKGSGYSFTSYWIGWVRQMPGKGLEWMGIIYPGDSDTRYSPSFQGQVTISADKSISTAYLQWSSLKASDTAMYYCARLSYSWSSWYWDFWGQGTLVTVSSGGGGSEIVLTQSPGTLSLSPGERATLSCRASQSVSSSYLAWYQQKPGQAPRLLIYGASSRATGIPDRFSGSGSGTDFTLTISRLEPEDFAVYYCQQAGLFPYTFGGGTKVEIKGSTSGSGKPGSGEGSTKGQVQLQESGPGLVKPSGTLSLTCAVSGGSISSSNWWSWVRQPPGKGLEWIGEIYHSGSTNYNPSLKSRVTISVDKSKNQFSLKLSSVTAADTAVYYCARLPGYESAFDIWGQGTMVTVSSGGGGSQAVLTQPPSVSEAPRQRVTISCSGSSSNIGNNAVSWYQQLPGKAPKLLIYYDDLLPSGVSDRFSGSKSGTSASLAISGLQSEDEADYYCAAWDDSLNGWVFGGGTKVTVLGFVPVFLPAKPTTTPAPRPPTPAPTIASQPLSLRPEACRPAAGGAVHTRGLDFACDIYIWAPLAGTCGVLLLSLVITLYCNHRNKRGRKKLLYIFKQPFMRPVQTTQEEDGCSCRFPEEEEGGCELRVKFSRSADAPAYQQGQNQLYNELNLGRREEYDVLDKRRGRDPEMGGKPRRKNPQEGLYNELQKDKMAEAYSEIGMKGERRRGKGHDGLYQGLSTATKDTYDALHMQALPPR

SEQ ID NO: 67 - DNA, 2235 bp, Artificial Sequence
  PXL1436 CAR nucleic acid sequence
atggcacttcctgtgacagccttgctcttgcccttagcactgctgcttcatgcggcgagacctgagatcgtcctcactcagtctccaggcaccctgtctttgtcacctggagaacgggcaacactttcatgcagagcatcacaaagcgttagtagtagctatcttgcctggtatcagcaaaaaccgggccaggcacctagactgctcatttatggagcttcctcaagagcaacaggaatccctgaccggttcagcgggtccggctctggtactgatttcaccttaacaatctcaagacttgaacctgaagatttcgcagtgtattattgtcagcaggcaggactcttcccgtatacattcggcggaggcacaaaagtggaaattaaaggagggggagggagcgaggtccaacttgtgcaatcaggagcagaagtgaagaagccaggcgaatcacttaagatttcctgcaaaggatcaggatactcatttacatcatactggatcggatgggtccggcagatgcccggcaaaggattggagtggatgggcatcatctaccctggagattcagatacaagatactcaccttccttccaaggccaggtcaccatatcggctgacaaatcaatctcaacagcataccttcaatggtcatcacttaaagcatcagatacagcaatgtactactgcgcaaggcttagctattcatggtcatcatggtactgggatttctgggggcaaggcacgctggttacagtctcatccggtagtacctccggatcaggaaagccgggctctggagaaggatctacaaagggccaagcagtactgacgcagccgccctcagtgtcagaggcgccaaggcaaagagtaaccataagttgttctggatcttccagcaatattggtaacaacgcagtgagctggtatcagcagctaccgggaaaggctcccaagctattgatatattatgacgatcttcttccttcaggagtgtcagacaggttctcgggttctaaatcaggcacatcagcatcacttgccatcagcggcctgcagagcgaagatgaagcagattattattgtgccgcgtgggatgattcacttaacggatgggtgttcggcggaggcacgaaggtgacagtacttggtggaggaggtggctcccaggttcaacttcaagaatccggcccaggtttggtaaagccttcaggtaccttatcgctgacttgtgcagtgtcaggaggatcaatctccagtagtaattggtggtcatgggtccgacagcctccagggaaaggactagagtggattggcgagatttaccactctgggagtaccaactacaacccttcacttaaatcacgagtcacaattagtgttgataaatcaaagaatcaattcagcctcaagctatcatcagtgacagcagcagatacagcggtctattattgtgctagacttccaggctacgaatcagcatttgatatctggggacaaggaaccatggtaactgttagtagctttgtacctgtgtttcttcctgcaaagccgaccacaactcccgcacctagacctccaactccggcaccaaccattgcatcacaacctctaagtctgaggcccgaggcatgcagacctgcagcaggaggagcagtgcacacaagaggacttgatttcgcgtgtgatatctacatctgggcacccctggccggaacatgtggagtgcttcttctttcacttgtgatcacactttactgcaaccacagaaacaagcgcggtagaaagaagctactgtacatctttaaacaacctttcatgcgtcctgtgcaaacaacacaagaagaagatggatgctcatgcagatttcctgaagaagaagaaggaggatgcgaacttagagtgaaattcagccgatcagcagatgcacctgcataccaacaaggacagaatcagctctataatgagctgaatttgggaagaagagaagaatacgatgtgcttgataagcgcagaggtcgagacccagaaatgggaggaaagccgaggaggaagaatccgcaagaaggactatataatgagctccagaaggataagatggctgaagcatactcagaaatcggaatgaaaggagaaagaagaagaggaaagggccatgatggactttaccaaggactttcaacagcaacaaaggacacttacgatgcacttcacatgcaagcacttcctcctaga

SEQ ID NO: 68 - protein, 745 aa, Artificial Sequence
  PXL1436 CAR protein sequence
MALPVTALLLPLALLLHAARPEIVLTQSPGTLSLSPGERATLSCRASQSVSSSYLAWYQQKPGQAPRLLIYGASSRATGIPDRFSGSGSGTDFTLTISRLEPEDFAVYYCQQAGLFPYTFGGGTKVEIKGGGGSEVQLVQSGAEVKKPGESLKISCKGSGYSFTSYWIGWVRQMPGKGLEWMGIIYPGDSDTRYSPSFQGQVTISADKSISTAYLQWSSLKASDTAMYYCARLSYSWSSWYWDFWGQGTLVTVSSGSTSGSGKPGSGEGSTKGQAVLTQPPSVSEAPRQRVTISCSGSSSNIGNNAVSWYQQLPGKAPKLLIYYDDLLPSGVSDRFSGSKSGTSASLAISGLQSEDEADYYCAAWDDSLNGWVFGGGTKVTVLGGGGGSQVQLQESGPGLVKPSGTLSLTCAVSGGSISSSNWWSWVRQPPGKGLEWIGEIYHSGSTNYNPSLKSRVTISVDKSKNQFSLKLSSVTAADTAVYYCARLPGYESAFDIWGQGTMVTVSSFVPVFLPAKPTTTPAPRPPTPAPTIASQPLSLRPEACRPAAGGAVHTRGLDFACDIYIWAPLAGTCGVLLLSLVITLYCNHRNKRGRKKLLYIFKQPFMRPVQTTQEEDGCSCRFPEEEEGGCELRVKFSRSADAPAYQQGQNQLYNELNLGRREEYDVLDKRRGRDPEMGGKPRRKNPQEGLYNELQKDKMAEAYSEIGMKGERRRGKGHDGLYQGLSTATKDTYDALHMQALPPR

SEQ ID NO: 69 - DNA, 2235 bp, Artificial Sequence
  PXL1437 CAR nucleic acid sequence
atggcacttcctgtgacagccttgctcttgcccttagcactgctgcttcatgcggcgagacctcaggttcaacttcaagaatccggcccaggtttggtaaagccttcaggtaccttatcgctgacttgtgcagtgtcaggaggatcaatctccagtagtaattggtggtcatgggtccgacagcctccagggaaaggactagagtggattggcgagatttaccactctgggagtaccaactacaacccttcacttaaatcacgagtcacaattagtgttgataaatcaaagaatcaattcagcctcaagctatcatcagtgacagcagcagatacagcggtctattattgtgctagacttccaggctacgaatcagcatttgatatctggggacaaggaaccatggtaactgttagtagcggagggggagggagccaagcagtactgacgcagccgccctcagtgtcagaggcgccaaggcaaagagtaaccataagttgttctggatcttccagcaatattggtaacaacgcagtgagctggtatcagcagctaccgggaaaggctcccaagctattgatatattatgacgatcttcttccttcaggagtgtcagacaggttctcgggttctaaatcaggcacatcagcatcacttgccatcagcggcctgcagagcgaagatgaagcagattattattgtgccgcgtgggatgattcacttaacggatgggtgttcggcggaggcacgaaggtgacagtacttggtggtagtacctccggatcaggaaagccgggctctggagaaggatctacaaagggcgaggtccaacttgtgcaatcaggagcagaagtgaagaagccaggcgaatcacttaagatttcctgcaaaggatcaggatactcatttacatcatactggatcggatgggtccggcagatgcccggcaaaggattggagtggatgggcatcatctaccctggagattcagatacaagatactcaccttccttccaaggccaggtcaccatatcggctgacaaatcaatctcaacagcataccttcaatggtcatcacttaaagcatcagatacagcaatgtactactgcgcaaggcttagctattcatggtcatcatggtactgggatttctgggggcaaggcacgctggttacagtctcatccggaggaggtggctccgagatcgtcctcactcagtctccaggcaccctgtctttgtcacctggagaacgggcaacactttcatgcagagcatcacaaagcgttagtagtagctatcttgcctggtatcagcaaaaaccgggccaggcacctagactgctcatttatggagcttcctcaagagcaacaggaatccctgaccggttcagcgggtccggctctggtactgatttcaccttaacaatctcaagacttgaacctgaagatttcgcagtgtattattgtcagcaggcaggactcttcccgtatacattcggcggaggcacaaaagtggaaattaaatttgtacctgtgtttcttcctgcaaagccgaccacaactcccgcacctagacctccaactccggcaccaaccattgcatcacaacctctaagtctgaggcccgaggcatgcagacctgcagcaggaggagcagtgcacacaagaggacttgatttcgcgtgtgatatctacatctgggcacccctggccggaacatgtggagtgcttcttctttcacttgtgatcacactttactgcaaccacagaaacaagcgcggtagaaagaagctactgtacatctttaaacaacctttcatgcgtcctgtgcaaacaacacaagaagaagatggatgctcatgcagatttcctgaagaagaagaaggaggatgcgaacttagagtgaaattcagccgatcagcagatgcacctgcataccaacaaggacagaatcagctctataatgagctgaatttgggaagaagagaagaatacgatgtgcttgataagcgcagaggtcgagacccagaaatgggaggaaagccgaggaggaagaatccgcaagaaggactatataatgagctccagaaggataagatggctgaagcatactcagaaatcggaatgaaaggagaaagaagaagaggaaagggccatgatggactttaccaaggactttcaacagcaacaaaggacacttacgatgcacttcacatgcaagcacttcctcctaga

SEQ ID NO: 70 - protein, 745 aa, Artificial Sequence
  PXL1437 CAR protein sequence
MALPVTALLLPLALLLHAARPQVQLQESGPGLVKPSGTLSLTCAVSGGSISSSNWWSWVRQPPGKGLEWIGEIYHSGSTNYNPSLKSRVTISVDKSKNQFSLKLSSVTAADTAVYYCARLPGYESAFDIWGQGTMVTVSSGGGGSQAVLTQPPSVSEAPRQRVTISCSGSSSNIGNNAVSWYQQLPGKAPKLLIYYDDLLPSGVSDRFSGSKSGTSASLAISGLQSEDEADYYCAAWDDSLNGWVFGGGTKVTVLGGSTSGSGKPGSGEGSTKGEVQLVQSGAEVKKPGESLKISCKGSGYSFTSYWIGWVRQMPGKGLEWMGIIYPGDSDTRYSPSFQGQVTISADKSISTAYLQWSSLKASDTAMYYCARLSYSWSSWYWDFWGQGTLVTVSSGGGGSEIVLTQSPGTLSLSPGERATLSCRASQSVSSSYLAWYQQKPGQAPRLLIYGASSRATGIPDRFSGSGSGTDFTLTISRLEPEDFAVYYCQQAGLFPYTFGGGTKVEIKFVPVFLPAKPTTTPAPRPPTPAPTIASQPLSLRPEACRPAAGGAVHTRGLDFACDIYIWAPLAGTCGVLLLSLVITLYCNHRNKRGRKKLLYIFKQPFMRPVQTTQEEDGCSCRFPEEEEGGCELRVKFSRSADAPAYQQGQNQLYNELNLGRREEYDVLDKRRGRDPEMGGKPRRKNPQEGLYNELQKDKMAEAYSEIGMKGERRRGKGHDGLYQGLSTATKDTYDALHMQALPPR